European Patent Application EP 4 790 068 A1, published August 12, 2026. Title: Neutralization of the pro-inflammatory effect of Bactericidal/permeability- increasing protein (BPI). Applicant: Universität Regensburg, in Vertretung des Freistaats Bayern. The sequence listing filed with the application follows.

SEQUENCE LISTING (153 sequences)

SEQ ID NO: 1 - protein, 15 aa, synthetic construct
FPAAHDRMVYLGLSD

SEQ ID NO: 2 - protein, 19 aa, synthetic construct
VYLGLSDYFFNTAGLVYQE

SEQ ID NO: 3 - protein, 19 aa, synthetic construct
PVMEFPAAHDRMVYLGLSD

SEQ ID NO: 4 - protein, 13 aa, synthetic construct
TFLPEVAKKFPNM

SEQ ID NO: 5 - protein, 22 aa, synthetic construct
FQTLPVMTKIDSVAGINYLVAP

SEQ ID NO: 6 - protein, 8 aa, synthetic construct
GFNFSTYG

SEQ ID NO: 7 - protein, 8 aa, synthetic construct
ISGGGSYT

SEQ ID NO: 8 - protein, 11 aa, synthetic construct
ARHENGPWFAY

SEQ ID NO: 9 - protein, 8 aa, synthetic construct
GFTFSIYD

SEQ ID NO: 10 - protein, 8 aa, synthetic construct
VSGGGSYT

SEQ ID NO: 11 - protein, 11 aa, synthetic construct
ARHENGPWFAY

SEQ ID NO: 12 - protein, 10 aa, synthetic construct
KSVSASDYSY

SEQ ID NO: 13 - skipped

SEQ ID NO: 14 - protein, 9 aa, synthetic construct
QHSRELPYT

SEQ ID NO: 15 - protein, 8 aa, synthetic construct
GFTFSTYG

SEQ ID NO: 16 - protein, 8 aa, synthetic construct
VSGGGTYT

SEQ ID NO: 17 - protein, 11 aa, synthetic construct
ARHETGPWFAY

SEQ ID NO: 18 - protein, 10 aa, synthetic construct
KSVSTSGYSY

SEQ ID NO: 19 - skipped

SEQ ID NO: 20 - protein, 9 aa, synthetic construct
QHSRELPYT

SEQ ID NO: 21 - protein, 8 aa, synthetic construct
GFSLISSA

SEQ ID NO: 22 - protein, 7 aa, synthetic construct
IWAGGST

SEQ ID NO: 23 - protein, 12 aa, synthetic construct
ATYYRFDDGFAY

SEQ ID NO: 24 - protein, 11 aa, synthetic construct
QSLVHSSGITY

SEQ ID NO: 25 - skipped

SEQ ID NO: 26 - protein, 9 aa, synthetic construct
SQSTHFPYT

SEQ ID NO: 27 - protein, 8 aa, synthetic construct
GFTFSNYG

SEQ ID NO: 28 - protein, 8 aa, synthetic construct
ISGGGNYT

SEQ ID NO: 29 - protein, 13 aa, synthetic construct
ARREAQLGSAMDY

SEQ ID NO: 30 - protein, 10 aa, synthetic construct
KSVSTSGYSY

SEQ ID NO: 31 - skipped

SEQ ID NO: 32 - protein, 9 aa, synthetic construct
QHSRELPLT

SEQ ID NO: 33 - protein, 8 aa, synthetic construct
GYEFSISW

SEQ ID NO: 34 - protein, 8 aa, synthetic construct
IFPGDGDT

SEQ ID NO: 35 - protein, 6 aa, synthetic construct
AREVGR

SEQ ID NO: 36 - protein, 6 aa, synthetic construct
QDIYNY

SEQ ID NO: 37 - skipped

SEQ ID NO: 38 - protein, 9 aa, synthetic construct
QQGNTLPYT

SEQ ID NO: 39 - protein, 6 aa, synthetic construct
QSIGTS

SEQ ID NO: 40 - skipped

SEQ ID NO: 41 - protein, 9 aa, synthetic construct
QQSNSWPLT

SEQ ID NO: 42 - protein, 8 aa, synthetic construct
GFDFDRYW

SEQ ID NO: 43 - protein, 8 aa, synthetic construct
INPNNNTI

SEQ ID NO: 44 - protein, 14 aa, synthetic construct
ARPGFYYGSAWFAY

SEQ ID NO: 45 - protein, 9 aa, synthetic construct
TGAVTTSNY

SEQ ID NO: 46 - skipped

SEQ ID NO: 47 - protein, 9 aa, synthetic construct
ALWYNSHWV

SEQ ID NO: 48 - protein, 8 aa, synthetic construct
GYTFTSYP

SEQ ID NO: 49 - protein, 8 aa, synthetic construct
FHPYNDDT

SEQ ID NO: 50 - protein, 10 aa, synthetic construct
ARAFYGNYDY

SEQ ID NO: 51 - protein, 6 aa, synthetic construct
QSVNND

SEQ ID NO: 52 - skipped

SEQ ID NO: 53 - protein, 9 aa, synthetic construct
HQNNRSPWT

SEQ ID NO: 54 - protein, 6 aa, synthetic construct
DHINNW

SEQ ID NO: 55 - skipped

SEQ ID NO: 56 - protein, 9 aa, synthetic construct
QQYWSSPYT

SEQ ID NO: 57 - protein, 8 aa, synthetic construct
GFTFSNYW

SEQ ID NO: 58 - protein, 10 aa, synthetic construct
IRLKSNNYAT

SEQ ID NO: 59 - protein, 9 aa, synthetic construct
TQSYYSMDY

SEQ ID NO: 60 - protein, 12 aa, synthetic construct
QSLLNSGNQKNY

SEQ ID NO: 61 - skipped

SEQ ID NO: 62 - protein, 9 aa, synthetic construct
QNDHSYPRT

SEQ ID NO: 63 - protein, 8 aa, synthetic construct
GFTFSNYW

SEQ ID NO: 64 - protein, 10 aa, synthetic construct
IRLKSNNYAT

SEQ ID NO: 65 - protein, 9 aa, synthetic construct
TQSYYSMDY

SEQ ID NO: 66 - protein, 12 aa, synthetic construct
QSLLYSSNQKNF

SEQ ID NO: 67 - skipped

SEQ ID NO: 68 - protein, 9 aa, synthetic construct
QQYYNYPYT

SEQ ID NO: 69 - protein, 8 aa, synthetic construct
GFTFSNYW

SEQ ID NO: 70 - protein, 10 aa, synthetic construct
IRLRSNNYAS

SEQ ID NO: 71 - protein, 9 aa, synthetic construct
AQSYYAMDY

SEQ ID NO: 72 - protein, 8 aa, synthetic construct
GFNIKDSY

SEQ ID NO: 73 - protein, 8 aa, synthetic construct
IDPANGDT

SEQ ID NO: 74 - protein, 8 aa, synthetic construct
ALYGYRAY

SEQ ID NO: 75 - protein, 12 aa, synthetic construct
QSLLNSGNQKNY

SEQ ID NO: 76 - skipped

SEQ ID NO: 77 - protein, 9 aa, synthetic construct
QNDHSYPRT

SEQ ID NO: 78 - protein, 118 aa, synthetic construct
EVKLVESGGDFVKPGGSLKLSCAASGFNFSTYGMSWVRQTPDKRLEWVATISGGGSYTFYLDSVKGRLTISRDNAKNTLYLQMSSLKSEDTAIYCCARHENGPWFAYWGQGTLVTVSA

SEQ ID NO: 79 - protein, 118 aa, synthetic construct
EVKLVESGGDFVKPGGSLKLSCAASGFTFSIYDMSWVRQTPDKRLEWVASVSGGGSYTFYPDSVKGRFTISRDNAKNTLYLQLSSLKSEDTAMYFCARHENGPWFAYWGQGTLVTVSA

SEQ ID NO: 80 - protein, 112 aa, synthetic construct
DIQLTQSPASLTISLGQRATISCRASKSVSASDYSYMHWYQQRSGQPPKLLIYLASNLDSGVPARFSGSGSGTDFTLNIHPVEEEDAATYYCQHSRELPYTFGGGTKLEVKR

SEQ ID NO: 81 - protein, 118 aa, synthetic construct
EVKLVESGGDFVKPGGSLKLSCAASGFTFSTYGMSWIRQTPDKRLEWVASVSGGGTYTFSPDSVKGRFTISRDSAKNTLYLQMSSLKSEDTAIYFCARHETGPWFAYWGQGTLVTVSA

SEQ ID NO: 82 - protein, 112 aa, synthetic construct
DIQMTQTPASLTISLGQRATISCRASKSVSTSGYSYMHWYRQKPGQPPKLLIYLASNLESGVPARFSGSGSGTDFTLNIHPVEEEDAATYYCQHSRELPYTFGGGTKLEIKR

SEQ ID NO: 83 - protein, 118 aa, synthetic construct
QVQLKESGPGLVAPSQSLSISCTVSGFSLISSAVHWVRQPPGKGLEWLGVIWAGGSTNYNSPLMSRLSISKDNSENQVFLKMNSLHSDDTAIYYCATYYRFDDGFAYWGQGTLVTVSA

SEQ ID NO: 84 - protein, 113 aa, synthetic construct
DIQMTQTPLSLPVSLGDQASISCRSSQSLVHSSGITYLHWYLQKPGQSPMVLIYRVSNRFSGVPDRFSGSGSGTDFTLKISRVEAEDLGVYFCSQSTHFPYTFGGGTKLEIKR

SEQ ID NO: 85 - protein, 120 aa, synthetic construct
EVKLVESGGGLVKPGGSLKLSCAASGFTFSNYGMSWVRQTPEKRLEWVATISGGGNYTFYPDNVRGRFTISRDNAKNNLYLQMSSLRSDDTALYYCARREAQLGSAMDYWGQGTSVTVSS

SEQ ID NO: 86 - protein, 111 aa, synthetic construct
DIVLTQSPASLAVSLGQRATISCRASKSVSTSGYSYMHWYQQKPGQPPKLLIYLASSLESGVPARFSGSGSGTDFTLNIHPVEEEDAATYYCQHSRELPLTFGAGTKLELK

SEQ ID NO: 87 - protein, 113 aa, synthetic construct
QVQLKESGPELVKPGASVKISCNASGYEFSISWMNWVRQRPGQGLEWIGRIFPGDGDTNYNGKFKGKATLTADKSSNTAYIHLNSLTSVDSAVYFCAREVGRWGQGTLVTVSP

SEQ ID NO: 88 - protein, 108 aa, synthetic construct
DIQMTQTTSSLSASLGDRVTISCRASQDIYNYLNWYQQKPDGTVELLIYYTSRLHSGVPSRFSGSGSGTDYSLTISNLEQEDIATYFCQQGNTLPYTFGGGTNLEIKR

SEQ ID NO: 89 - protein, 107 aa, synthetic construct
DIQLTQSPAILSVSPGERVSFSCRASQSIGTSIHWYQQRTNGSPRLLIKYASDSISGIPSRFSGSGSGTDFTLSINSVESEDIADYYCQQSNSWPLTFGAGTKLELK

SEQ ID NO: 90 - protein, 121 aa, synthetic construct
EVKLVESGGGLVQPGGSLKLSCSASGFDFDRYWMSWVRQAPGKGLEWIGEINPNNNTINYTPSLTDKFIISRDNAKNTLYLQMSKVSSEDTALYYCARPGFYYGSAWFAYWGQGTLVTVSA

SEQ ID NO: 91 - protein, 109 aa, synthetic construct
QAVVTQESALTTSPGETVTLTCRSSTGAVTTSNYANWVQEKPDHLFTGLIGGSNNRAPGIPARFSGFLIGDKAALTITGAQTEDEAIYFCALWYNSHWVFGGGTKLTVL

SEQ ID NO: 92 - protein, 117 aa, synthetic construct
EVKLVESGAELVKPGASVKMSCKASGYTFTSYPLEWMKQSHGMSLEWIGNFHPYNDDTKSNDKFAGKATLTVEKSSSTVYLELSRLTSDDSAVYFCARAFYGNYDYWGQGTTLTVSS

SEQ ID NO: 93 - protein, 107 aa, synthetic construct
DIQMTQTPKFLLVSAGDRVTILCKASQSVNNDVGWYQQRPGQSPKLLIYYASTRYTGVPDRFTGSGYGTDFTFTINSVQAEDLALYFCHQNNRSPWTFGGGTKLEIK

SEQ ID NO: 94 - protein, 108 aa, synthetic construct
DIQMTQTSSYLSVSLGDRVTITCKASDHINNWLAWYQQKPGNAPRLLISGTTSLENGDPSRFSGSGSGRDYTLSISSLQTEDVATYYCQQYWSSPYTFGGGTKLEIIR

SEQ ID NO: 95 - protein, 118 aa, synthetic construct
EVKLVESGGGLVQPGGSMKLSCVASGFTFSNYWMDWVRQSPEKGLEWVAEIRLKSNNYATHYAESVKGRFTISRDDSKSSVYLQMNNLRAEDTGIYYCTQSYYSMDYWGQGTSVTVSS

SEQ ID NO: 96 - protein, 113 aa, synthetic construct
DILMTQSPSSLSVSTGEKVTMSCKSSQSLLNSGNQKNYLAWYQQKPGQPPKLLIYGASTRDSGVPNRFTGSGSGTDFSLTISSVQAEDLAVYYCQNDHSYPRTFGGGTKLEIK

SEQ ID NO: 97 - protein, 118 aa, synthetic construct
DVKLQESGGGLVQPGRSMKLSCVASGFTFSNYWMDWVRQSPEKGLEWVAEIRLKSNNYATHYAESVKGRFTISRDDSKSSVYLQMNNLKTEDTGIYYCTQSYYSMDYWGQGTSVTVSS

SEQ ID NO: 98 - protein, 114 aa, synthetic construct
DIVMTQSPSSLAVSVGEKVTMSCKSSQSLLYSSNQKNFLAWYQQKPGQSPKLLIYWASTRESGVPDRFTGSGSGTDFTLTISSVKAEDLAVYYCQQYYNYPYTFGGGTKLEIKR

SEQ ID NO: 99 - protein, 118 aa, synthetic construct
EVKLVESGGGLVQPGGSMKLSCVASGFTFSNYWMNWVRQSPEKGLEWVAEIRLRSNNYASYYAESVRGRFTISRDDSKSSVYLQMNNLRAEDTGIYYCAQSYYAMDYWGQGTSVTVSS

SEQ ID NO: 100 - protein, 115 aa, synthetic construct
EVKLVESGAELVKPGASVKLSCTASGFNIKDSYIHWVKQRPEQGLEWIGRIDPANGDTKYDPKFQGKATITADTSSNTAYLQLSSLTSEDTAVYYCALYGYRAYWGQGTLVTVSA

SEQ ID NO: 101 - protein, 113 aa, synthetic construct; identical to SEQ ID NO: 96

SEQ ID NO: 102 - protein, 15 aa, synthetic construct
HYSFYSMDIREFQLP

SEQ ID NO: 103 - protein, 19 aa, synthetic construct
MVPNVGLKFSISNANIKIS

SEQ ID NO: 104 - protein, 15 aa, synthetic construct
QKRFLKMSGNFDLSI

SEQ ID NO: 105 - protein, 466 aa, Homo sapiens
VNPGVVVRVSQKGLDYASQQGTAALQKELKRIKIPDYSDSFKIKHLGKGHYSFYSMDIREFQLPSSQISMVPNVGLKFSISNANIKISGKWKAQKRFLKMSGNFDLSIEGMSISADLKLGSNPTSGKPTITCSSCSSHINSVHVHISKSKVGWLIQLFHKKIESALRNKMNSQVCEKVTNSVSSELQPYFQTLPVMTKIDSVAGINYGLVAPPATTAETLDVQMKGEFYSENHHNPPPFAPPVMEFPAAHDRMVYLGLSDYFFNTAGLVYQEAGVLKMTLRDDMIPKESKFRLTTKFFGTFLPEVAKKFPNMKIQIHVSASTPPHLSVQPTGLTFYPAVDVQAFAVLPNSSLASLFLIGMHTTGSMEVSAESNRLVGELKLDRLLLELKHSNIGPFPVELLQDIMNYIVPILVLPRVNEKLQKGFPLPTPARVQLYNVVLQPHQNFLLFGADVVYKQFDYKDDDDK

SEQ ID NO: 106 - protein, 466 aa, Mus musculus
TDPGFVAMISQKGLDFACQQGVVELQKELQAISVPDFSGVFKIKHLGKGSYEFYSMAVDGFHIPNPKIEMLPSDGLRVFIKDASIKINGKWMSRKNFLKAGGNFELSIQGVSISTDLILGSDSSGHITTICSNCDSHIDSVHIKISGSMLGWLIRLFHRKIETSLKNIIYKKICKIVRDSVSSKLQPYLKTLSVITRVDDVTSVDYSLLAPLTTTNQFLEGQLKGEFFWRGHRDPLPIHPPVMRFVPNGAYMVCMGISDYFFNTEVLAYQQSGTLKMTLGGQLLSNNGRFQLNTDFLRTFLPKVAKMFPSMGVQLLISAPVPVHLSIQPSGLSFNPKLETQAFVVLPNASLVPLFVLGMKTNASLEVDAEENRLVGEMKLGSRWLLELKESKFGPFKVEYLEDVINYLVSTLVLPKINERLRRGFPLPLPAGIRFSHFTFYPYQNFLLLEADLHLIQFDYKDDDDK

SEQ ID NO: 107 - protein, 59 aa, synthetic construct
QVQLKESGPGLVAPSQSLSISCTVSGFSLISSAVHWVRQPPGKGLEWLGVIWAGGSTNY

SEQ ID NO: 108 - protein, 60 aa, synthetic construct
EVKLVESGGGLVKPGGSLKLSCAASGFTFSNYGMSWVRQTPEKRLEWVATISGGGNYTFY

SEQ ID NO: 109 - protein, 60 aa, synthetic construct
EVKLVESGGDFVKPGGSLKLSCAASGFNFSTYGMSWVRQTPDKRLEWVATISGGGSYTFY

SEQ ID NO: 110 - protein, 60 aa, synthetic construct
EVKLVESGGDFVKPGGSLKLSCAASGFTFSIYDMSWVRQTPDKRLEWVASVSGGGSYTFY

SEQ ID NO: 111 - protein, 60 aa, synthetic construct
EVKLVESGGDFVKPGGSLKLSCAASGFTFSTYGMSWIRQTPDKRLEWVASVSGGGTYTFS

SEQ ID NO: 112 - protein, 59 aa, synthetic construct
NSPLMSRLSISKDNSENQVFLKMNSLHSDDTAIYYCATYYRFDDGFAYWGQGTLVTVSA

SEQ ID NO: 113 - protein, 60 aa, synthetic construct
PDNVRGRFTISRDNAKNNLYLQMSSLRSDDTALYYCARREAQLGSAMDYWGQGTSVTVSS

SEQ ID NO: 114 - protein, 58 aa, synthetic construct
LDSVKGRLTISRDNAKNTLYLQMSSLKSEDTAIYCCARHENGPWFAYWGQGTLVTVSA

SEQ ID NO: 115 - protein, 58 aa, synthetic construct
PDSVKGRFTISRDNAKNTLYLQLSSLKSEDTAMYFCARHENGPWFAYWGQGTLVTVSA

SEQ ID NO: 116 - protein, 58 aa, synthetic construct
PDSVKGRFTISRDSAKNTLYLQMSSLKSEDTAIYFCARHETGPWFAYWGQGTLVTVSA

SEQ ID NO: 117 - protein, 55 aa, synthetic construct
DIQLTQSPAILSVSPGERVSFSCRASQSIGTSIHWYQQRTNGSPRLLIKYASDSI

SEQ ID NO: 118 - protein, 60 aa, synthetic construct
DIQMTQTPLSLPVSLGDQASISCRSSQSLVHSSGITYLHWYLQKPGQSPMVLIYRVSNRF

SEQ ID NO: 119 - protein, 59 aa, synthetic construct
DIVLTQSPASLAVSLGQRATISCRASKSVSTSGYSYMHWYQQKPGQPPKLLIYLASSLE

SEQ ID NO: 120 - protein, 59 aa, synthetic construct
DIQLTQSPASLTISLGQRATISCRASKSVSASDYSYMHWYQQRSGQPPKLLIYLASNLD

SEQ ID NO: 121 - protein, 59 aa, synthetic construct
DIQMTQTPASLTISLGQRATISCRASKSVSTSGYSYMHWYRQKPGQPPKLLIYLASNLE

SEQ ID NO: 122 - protein, 52 aa, synthetic construct
SGIPSRFSGSGSGTDFTLSINSVESEDIADYYCQQSNSWPLTFGAGTKLELK

SEQ ID NO: 123 - protein, 53 aa, synthetic construct
SGVPDRFSGSGSGTDFTLKISRVEAEDLGVYFCSQSTHFPYTFGGGTKLEIKR

SEQ ID NO: 124 - protein, 52 aa, synthetic construct
SGVPARFSGSGSGTDFTLNIHPVEEEDAATYYCQHSRELPLTFGAGTKLELK

SEQ ID NO: 125 - protein, 53 aa, synthetic construct
SGVPARFSGSGSGTDFTLNIHPVEEEDAATYYCQHSRELPYTFGGGTKLEVKR

SEQ ID NO: 126 - protein, 53 aa, synthetic construct
SGVPARFSGSGSGTDFTLNIHPVEEEDAATYYCQHSRELPYTFGGGTKLEIKR

SEQ ID NO: 127 - protein, 15 aa, synthetic construct
VYLGLSDYFFNTAGL

SEQ ID NO: 128 - protein, 15 aa, synthetic construct
LSDYFFNTAGLVYQE

SEQ ID NO: 129 - protein, 15 aa, synthetic construct
PVMEFPAAHDRMVYL

SEQ ID NO: 130 - protein, 15 aa, synthetic construct
FPAAHDRMVYLGLSD

SEQ ID NO: 131 - protein, 60 aa, synthetic construct
EVKLVESGGGLVQPGGSMKLSCVASGFTFSNYWMNWVRQSPEKGLEWVAEIRLRSNNYAS

SEQ ID NO: 132 - protein, 60 aa, synthetic construct
EVKLVESGGGLVQPGGSMKLSCVASGFTFSNYWMDWVRQSPEKGLEWVAEIRLKSNNYAT

SEQ ID NO: 133 - protein, 60 aa, synthetic construct
DVKLQESGGGLVQPGRSMKLSCVASGFTFSNYWMDWVRQSPEKGLEWVAEIRLKSNNYAT

SEQ ID NO: 134 - protein, 58 aa, synthetic construct
YYAESVRGRFTISRDDSKSSVYLQMNNLRAEDTGIYYCAQSYYAMDYWGQGTSVTVSS

SEQ ID NO: 135 - protein, 58 aa, synthetic construct
HYAESVKGRFTISRDDSKSSVYLQMNNLRAEDTGIYYCTQSYYSMDYWGQGTSVTVSS

SEQ ID NO: 136 - protein, 58 aa, synthetic construct
HYAESVKGRFTISRDDSKSSVYLQMNNLKTEDTGIYYCTQSYYSMDYWGQGTSVTVSS

SEQ ID NO: 137 - protein, 60 aa, synthetic construct
DILMTQSPSSLSVSTGEKVTMSCKSSQSLLNSGNQKNYLAWYQQKPGQPPKLLIYGASTR

SEQ ID NO: 138 - protein, 60 aa, synthetic construct
DIVMTQSPSSLAVSVGEKVTMSCKSSQSLLYSSNQKNFLAWYQQKPGQSPKLLIYWASTR

SEQ ID NO: 139 - protein, 53 aa, synthetic construct
DSGVPNRFTGSGSGTDFSLTISSVQAEDLAVYYCQNDHSYPRTFGGGTKLEIK

SEQ ID NO: 140 - protein, 54 aa, synthetic construct
ESGVPDRFTGSGSGTDFTLTISSVKAEDLAVYYCQQYYNYPYTFGGGTKLEIKR

SEQ ID NO: 141 - protein, 15 aa, synthetic construct
HYSFYSMDIREFQLP

SEQ ID NO: 142 - protein, 15 aa, synthetic construct
MVPNVGLKFSISNAN

SEQ ID NO: 143 - protein, 15 aa, synthetic construct
VGLKFSISNANIKIS

SEQ ID NO: 144 - protein, 15 aa, synthetic construct
QKRFLKMSGNFDLSI

SEQ ID NO: 145 - protein, 60 aa, synthetic construct
FLRTFLPKVAKMFPSMGVQLLISAPVPVHLSIQPSGLSFNPKLETQAFVVLPNASLVPLF

SEQ ID NO: 146 - protein, 60 aa, synthetic construct
FFGTFLPEVAKKFPNMKIQIHVSASTPPHLSVQPTGLTFYPAVDVQAFAVLPNSSLASLF

SEQ ID NO: 147 - protein, 15 aa, synthetic construct
FQTLPVMTKIDSVAG

SEQ ID NO: 148 - protein, 15 aa, synthetic construct
PVMTKIDSVAGINYG

SEQ ID NO: 149 - protein, 15 aa, synthetic construct
KIDSVAGINYGLVAP

SEQ ID NO: 150 - protein, 8 aa, synthetic construct
GFXFSXYX

SEQ ID NO: 151 - protein, 8 aa, synthetic construct
XSGGGXYT

SEQ ID NO: 152 - protein, 11 aa, synthetic construct
ARHEXGPWFAY

SEQ ID NO: 153 - protein, 10 aa, synthetic construct
KSVSXSXYSY